European Patent Specification EP 4 162 034 B1, published July 29, 2026. Title: RNA replicon for versatile and efficient gene expression. Applicant: BioNTech RNA Pharmaceuticals et al. The sequence listing filed with the application follows.

SEQUENCE LISTING (2 sequences)

SEQ ID NO: 1 - DNA, 21 bp, Artificial Sequence
  Primer
cacgttgacatcgaggaagac

SEQ ID NO: 2 - DNA, 20 bp, Artificial Sequence
  Primer
tccacctccgtttcgatcag